European Patent Application EP 4 129 321 A1, published February 8, 2023. Title: Composition. Applicant: Nuritas. The sequence listing filed with the application follows.

SEQUENCE LISTING (85 sequences)

SEQ ID NO: 1 - protein, 11 aa, Artificial Sequence
  Peptide
WKDEAGKPLVK

SEQ ID NO: 2 - protein, 11 aa, Artificial Sequence
  Peptide
WKEEAGKPLVK

SEQ ID NO: 3 - protein, 11 aa, Artificial Sequence
  Peptide
FKDEAGKPLVK

SEQ ID NO: 4 - protein, 11 aa, Artificial Sequence
  Peptide
WKDEAGKPMVK

SEQ ID NO: 5 - protein, 11 aa, Artificial Sequence
  Peptide
WKDEAGRPLVK

SEQ ID NO: 6 - protein, 11 aa, Artificial Sequence
  Peptide
WRDEAGKPLVK

SEQ ID NO: 7 - protein, 11 aa, Artificial Sequence
  Peptide
WKDEAGKPLMK

SEQ ID NO: 8 - protein, 11 aa, Artificial Sequence
  Peptide
WKDQAGKPLVK

SEQ ID NO: 9 - protein, 11 aa, Artificial Sequence
  Peptide
WKDEATKPLVK

SEQ ID NO: 10 - protein, 11 aa, Artificial Sequence
  Peptide
YKNEAGKPLVK

SEQ ID NO: 11 - protein, 11 aa, Artificial Sequence
  Peptide
WKNESGKPLVK

SEQ ID NO: 12 - protein, 11 aa, Artificial Sequence
  Peptide
WKDEAGKTLVR

SEQ ID NO: 13 - protein, 11 aa, Artificial Sequence
  Peptide
FKDEATKPLVK

SEQ ID NO: 14 - protein, 11 aa, Artificial Sequence
  Peptide
FKDEAGKPLIK

SEQ ID NO: 15 - protein, 11 aa, Artificial Sequence
  Peptide
WKDEAGKTLLK

SEQ ID NO: 16 - protein, 11 aa, Artificial Sequence
  Peptide
WKNEAGKPVVK

SEQ ID NO: 17 - protein, 11 aa, Artificial Sequence
  Peptide
WKDEAGRTLVK

SEQ ID NO: 18 - protein, 11 aa, Artificial Sequence
  Peptide
WEDESGKPLLK

SEQ ID NO: 19 - protein, 11 aa, Artificial Sequence
  Peptide
WKEEAGKPIVQ

SEQ ID NO: 20 - protein, 11 aa, Artificial Sequence
  Peptide
YKNEAGKPLVR

SEQ ID NO: 21 - protein, 11 aa, Artificial Sequence
  Peptide
WKDQATRPLVK

SEQ ID NO: 22 - protein, 11 aa, Artificial Sequence
  Peptide
WKDESGKPVLK

SEQ ID NO: 23 - protein, 11 aa, Artificial Sequence
  Peptide
WQDDSGKPLVK

SEQ ID NO: 24 - protein, 11 aa, Artificial Sequence
  Peptide
WKNEAGKTLLK

SEQ ID NO: 25 - protein, 11 aa, Artificial Sequence
  Peptide
WKDKAGEPLVR

SEQ ID NO: 26 - protein, 11 aa, Artificial Sequence
  Peptide
WKDEAGNPLVK

SEQ ID NO: 27 - protein, 11 aa, Artificial Sequence
  Peptide
CKDEAGKPLVK

SEQ ID NO: 28 - protein, 11 aa, Artificial Sequence
  Peptide
WKDEAGKPLGK

SEQ ID NO: 29 - protein, 11 aa, Artificial Sequence
  Peptide
WKDENGKPLVK

SEQ ID NO: 30 - protein, 11 aa, Artificial Sequence
  Peptide
WKDEARKPLVK

SEQ ID NO: 31 - protein, 11 aa, Artificial Sequence
  Peptide
WKDEAGKPLVT

SEQ ID NO: 32 - protein, 11 aa, Artificial Sequence
  Peptide
WKDEAGKRLVK

SEQ ID NO: 33 - protein, 11 aa, Artificial Sequence
  Peptide
WKWEAGKPLVK

SEQ ID NO: 34 - protein, 11 aa, Artificial Sequence
  Peptide
WKDEAGFPTVK

SEQ ID NO: 35 - protein, 11 aa, Artificial Sequence
  Peptide
WYDMAGKPLVK

SEQ ID NO: 36 - protein, 11 aa, Artificial Sequence
  Peptide
WKDYEGKPLVK

SEQ ID NO: 37 - protein, 11 aa, Artificial Sequence
  Peptide
WKREAGKPGVK

SEQ ID NO: 38 - protein, 11 aa, Artificial Sequence
  Peptide
WKLEKGKPLVK

SEQ ID NO: 39 - protein, 11 aa, Artificial Sequence
  Peptide
WKDEAGKPCVK

SEQ ID NO: 40 - protein, 11 aa, Artificial Sequence
  Peptide
WKKEAPKPLVK

SEQ ID NO: 41 - protein, 11 aa, Artificial Sequence
  Peptide
SKDEAGPPLVK

SEQ ID NO: 42 - protein, 11 aa, Artificial Sequence
  Peptide
WKHEPGKPLAK

SEQ ID NO: 43 - protein, 11 aa, Artificial Sequence
  Peptide
WKDEREKPFVK

SEQ ID NO: 44 - protein, 11 aa, Artificial Sequence
  Peptide
WKQEAGKPWRK

SEQ ID NO: 45 - protein, 11 aa, Artificial Sequence
  Peptide
VKDEAKKPLVH

SEQ ID NO: 46 - protein, 11 aa, Artificial Sequence
  Peptide
NWDEAGKMLVK

SEQ ID NO: 47 - protein, 11 aa, Artificial Sequence
  Peptide
IKDEDGPPLVK

SEQ ID NO: 48 - protein, 11 aa, Artificial Sequence
  Peptide
LKDEYGKPLVN

SEQ ID NO: 49 - protein, 11 aa, Artificial Sequence
  Peptide
WKDRAGKELTK

SEQ ID NO: 50 - protein, 12 aa, Artificial Sequence
  Peptide
WKDEAGKPLPVK

SEQ ID NO: 51 - protein, 14 aa, Artificial Sequence
  Peptide
WKGDENYAGKPLVK

SEQ ID NO: 52 - protein, 14 aa, Artificial Sequence
  Peptide
LWKDEAGRKYPLVK

SEQ ID NO: 53 - protein, 12 aa, Artificial Sequence
  Peptide
WKDCEGAGKPLV

SEQ ID NO: 54 - protein, 13 aa, Artificial Sequence
  Peptide
WKDEPAGKPLVVK

SEQ ID NO: 55 - protein, 12 aa, Artificial Sequence
  Peptide
WKDEAGPKPLVK

SEQ ID NO: 56 - protein, 14 aa, Artificial Sequence
  Peptide
WKDEAGWADKPLVK

SEQ ID NO: 57 - protein, 12 aa, Artificial Sequence
  Peptide
WKNDEAGKPLVK

SEQ ID NO: 58 - protein, 9 aa, Artificial Sequence
  Peptide
WKDAKPLVK

SEQ ID NO: 59 - protein, 9 aa, Artificial Sequence
  Peptide
WKEAGKPVK

SEQ ID NO: 60 - protein, 10 aa, Artificial Sequence
  Peptide
WKDEAKPLVK

SEQ ID NO: 61 - protein, 8 aa, Artificial Sequence
  Peptide
WDEAGKPV

SEQ ID NO: 62 - protein, 10 aa, Artificial Sequence
  Peptide
WKDEAGKPVK

SEQ ID NO: 63 - protein, 9 aa, Artificial Sequence
  Peptide
WDAGKPLVK

SEQ ID NO: 64 - protein, 10 aa, Artificial Sequence
  Peptide
WKDEAGKPLV

SEQ ID NO: 65 - protein, 8 aa, Artificial Sequence
  Peptide
WEAGKPLV

SEQ ID NO: 66 - protein, 6 aa, Artificial Sequence
  Peptide
WKDEAG

SEQ ID NO: 67 - protein, 5 aa, Artificial Sequence
  Peptide
WKDEA

SEQ ID NO: 68 - protein, 8 aa, Artificial Sequence
  Peptide
KDEAGKPL

SEQ ID NO: 69 - protein, 5 aa, Artificial Sequence
  Peptide
KDEAG

SEQ ID NO: 70 - protein, 7 aa, Artificial Sequence
  Peptide
DEAGKPL

SEQ ID NO: 71 - protein, 5 aa, Artificial Sequence
  Peptide
GKPLV

SEQ ID NO: 72 - protein, 5 aa, Artificial Sequence
  Peptide
DEAGK

SEQ ID NO: 73 - protein, 9 aa, Artificial Sequence
  Peptide
WKDEAGKPL

SEQ ID NO: 74-75 - skipped (2 entries)

SEQ ID NO: 76 - protein, 5 aa, Artificial Sequence
  Peptide
KPLVK

SEQ ID NO: 77 - protein, 4 aa, Artificial Sequence
  Peptide
WKDE

SEQ ID NO: 78 - protein, 5 aa, Artificial Sequence
  Peptide
AGKPL

SEQ ID NO: 79-85 - skipped (7 entries)